European Patent Application EP 4 553 087 A1, published May 14, 2025. Title: Novel TCTP Binding Molecules. Applicant: Boostimmune, Inc. Application WO. The sequence listing filed with the application follows.

SEQUENCE LISTING (178 sequences)

SEQ ID NO: 1 - protein, 5 aa, synthetic construct
GYYMH

SEQ ID NO: 2 - protein, 17 aa, synthetic construct
WINPNSGGTNYAQKFQG

SEQ ID NO: 3 - protein, 10 aa, synthetic construct
GITGTTPFDY

SEQ ID NO: 4 - protein, 11 aa, synthetic construct
RASQGIRNDLG

SEQ ID NO: 5 - protein, 7 aa, synthetic construct
AASSLQS

SEQ ID NO: 6 - protein, 9 aa, synthetic construct
LQHNSYPYT

SEQ ID NO: 7 - protein, 7 aa, synthetic construct
NARMGVS

SEQ ID NO: 8 - protein, 16 aa, synthetic construct
HIFSNDEKSYSTSLKS

SEQ ID NO: 9 - protein, 12 aa, synthetic construct
VLLWFGELYFDY

SEQ ID NO: 10 - protein, 11 aa, synthetic construct
RASQSVSSNLA

SEQ ID NO: 11 - protein, 7 aa, synthetic construct
GASTRAT

SEQ ID NO: 12 - protein, 9 aa, synthetic construct
QQYNNWPRT

SEQ ID NO: 13 - protein, 5 aa, synthetic construct
GYYMH

SEQ ID NO: 14 - protein, 17 aa, synthetic construct
WINPNSGGTNYAQKFQG

SEQ ID NO: 15 - protein, 11 aa, synthetic construct
LGTTGYYYFDY

SEQ ID NO: 16 - protein, 11 aa, synthetic construct
RASQSIGSSLH

SEQ ID NO: 17 - protein, 7 aa, synthetic construct
YASQSFS

SEQ ID NO: 18 - protein, 9 aa, synthetic construct
HQSSSLPRT

SEQ ID NO: 19 - protein, 5 aa, synthetic construct
SNAMH

SEQ ID NO: 20 - protein, 17 aa, synthetic construct
WINAGNGNTKYSQKFQG

SEQ ID NO: 21 - protein, 17 aa, synthetic construct
GYYDILTGYYTTDAFDI

SEQ ID NO: 22 - protein, 16 aa, synthetic construct
RSSQSLVYSDGNTYLN

SEQ ID NO: 23 - protein, 7 aa, synthetic construct
KVSNRDS

SEQ ID NO: 24 - protein, 9 aa, synthetic construct
MQGTHWPYT

SEQ ID NO: 25 - protein, 5 aa, synthetic construct
SYAMH

SEQ ID NO: 26 - protein, 17 aa, synthetic construct
WINAGNGYTEYSQKFQG

SEQ ID NO: 27 - protein, 11 aa, synthetic construct
RGYFDWWAFDY

SEQ ID NO: 28 - protein, 11 aa, synthetic construct
RASQSIGSSLH

SEQ ID NO: 29 - protein, 7 aa, synthetic construct
YASQSFS

SEQ ID NO: 30 - protein, 9 aa, synthetic construct
HQSSSLPQT

SEQ ID NO: 31 - protein, 6 aa, synthetic construct
SSNWWS

SEQ ID NO: 32 - protein, 16 aa, synthetic construct
EIDHSGTTTYNPSLKS

SEQ ID NO: 33 - protein, 9 aa, synthetic construct
DGSGSYEGY

SEQ ID NO: 34 - protein, 11 aa, synthetic construct
RASQAISNHLA

SEQ ID NO: 35 - protein, 7 aa, synthetic construct
AASSLQS

SEQ ID NO: 36 - protein, 9 aa, synthetic construct
QQYHSYPIT

SEQ ID NO: 37 - protein, 6 aa, synthetic construct
SSNWWS

SEQ ID NO: 38 - protein, 15 aa, synthetic construct
EIYHGVTTYNPSLKS

SEQ ID NO: 39 - protein, 9 aa, synthetic construct
DGSGSYEGY

SEQ ID NO: 40 - protein, 11 aa, synthetic construct
RASQDISNYLA

SEQ ID NO: 41 - protein, 7 aa, synthetic construct
AASSLQS

SEQ ID NO: 42 - protein, 9 aa, synthetic construct
QQYHYYPIT

SEQ ID NO: 43 - protein, 5 aa, synthetic construct
SYAMH

SEQ ID NO: 44 - protein, 17 aa, synthetic construct
WINAGNGNTKYSQKFQD

SEQ ID NO: 45 - protein, 5 aa, synthetic construct
WVFDY

SEQ ID NO: 46 - protein, 16 aa, synthetic construct
RSSQSLVHRDGNTYLS

SEQ ID NO: 47 - protein, 7 aa, synthetic construct
KISNRFF

SEQ ID NO: 48 - protein, 9 aa, synthetic construct
MQATQFPHT

SEQ ID NO: 49 - protein, 7 aa, synthetic construct
SNSAAWN

SEQ ID NO: 50 - protein, 18 aa, synthetic construct
RTYYRSKWYNDYAVSVKS

SEQ ID NO: 51 - protein, 15 aa, synthetic construct
EGITVGRGVMLYFDL

SEQ ID NO: 52 - protein, 16 aa, synthetic construct
RSSQSLVYSDGNTHLK

SEQ ID NO: 53 - protein, 7 aa, synthetic construct
KVSKWDS

SEQ ID NO: 54 - protein, 9 aa, synthetic construct
MQGTHWPPT

SEQ ID NO: 55 - protein, 10 aa, synthetic construct
GYTFTGYYMH

SEQ ID NO: 56 - protein, 17 aa, synthetic construct
WINPNSGGTNYAQKFQG

SEQ ID NO: 57 - protein, 11 aa, synthetic construct
PAPRLRGAFDI

SEQ ID NO: 58 - protein, 13 aa, synthetic construct
SGSSSNIGNKKVS

SEQ ID NO: 59 - protein, 7 aa, synthetic construct
DDNKRPS

SEQ ID NO: 60 - protein, 10 aa, synthetic construct
ATWDSSLRAV

SEQ ID NO: 61 - protein, 5 aa, synthetic construct
SHAVH

SEQ ID NO: 62 - protein, 17 aa, synthetic construct
WINAGKGNTKYSQKFQG

SEQ ID NO: 63 - protein, 8 aa, synthetic construct
GRAVAFDP

SEQ ID NO: 64 - protein, 14 aa, synthetic construct
TGTNSDIGGYNYVS

SEQ ID NO: 65 - protein, 7 aa, synthetic construct
EVNKRPS

SEQ ID NO: 66 - protein, 10 aa, synthetic construct
ASYAGDNNLV

SEQ ID NO: 67 - protein, 7 aa, synthetic construct
SNSAAWN

SEQ ID NO: 68 - protein, 18 aa, synthetic construct
RTYYRSKWYNDYAVSVKS

SEQ ID NO: 69 - protein, 8 aa, synthetic construct
GGAAVFDY

SEQ ID NO: 70 - protein, 17 aa, synthetic construct
KSSQSILYNSNNKNYLA

SEQ ID NO: 71 - protein, 7 aa, synthetic construct
WASTRGS

SEQ ID NO: 72 - protein, 9 aa, synthetic construct
QQYYSTPLT

SEQ ID NO: 73 - protein, 5 aa, synthetic construct
GYYMH

SEQ ID NO: 74 - protein, 17 aa, synthetic construct
WINPNSGDTNYAQKFQG

SEQ ID NO: 75 - protein, 15 aa, synthetic construct
GGVLLYFGELSRFDY

SEQ ID NO: 76 - protein, 14 aa, synthetic construct
TGTSSDVGGYNYVS

SEQ ID NO: 77 - protein, 7 aa, synthetic construct
EVTKRPS

SEQ ID NO: 78 - protein, 10 aa, synthetic construct
ASYAGDNNLV

SEQ ID NO: 79 - protein, 5 aa, synthetic construct
VNAMH

SEQ ID NO: 80 - protein, 17 aa, synthetic construct
WINAGTGKTKYSQKFQG

SEQ ID NO: 81 - protein, 8 aa, synthetic construct
GRAVAFDP

SEQ ID NO: 82 - protein, 14 aa, synthetic construct
TGTSSDVGGYDYVS

SEQ ID NO: 83 - protein, 7 aa, synthetic construct
EVNKRPS

SEQ ID NO: 84 - protein, 10 aa, synthetic construct
NSYAGNNNLV

SEQ ID NO: 85 - protein, 7 aa, synthetic construct
SNSAAWN

SEQ ID NO: 86 - protein, 18 aa, synthetic construct
RTYYKSKWYNDYAVSVKS

SEQ ID NO: 87 - protein, 8 aa, synthetic construct
GGSAVFDY

SEQ ID NO: 88 - protein, 17 aa, synthetic construct
KSSQSILYSSNNKNYLA

SEQ ID NO: 89 - protein, 7 aa, synthetic construct
WASTRKS

SEQ ID NO: 90 - protein, 9 aa, synthetic construct
QQYYGLPLT

SEQ ID NO: 91 - protein, 7 aa, synthetic construct
SNSAAWN

SEQ ID NO: 92 - protein, 18 aa, synthetic construct
RTYYKSKWYNDYAVSVKS

SEQ ID NO: 93 - protein, 8 aa, synthetic construct
GGSAVFDY

SEQ ID NO: 94 - protein, 17 aa, synthetic construct
KSSQSVLYSSNNKNYLA

SEQ ID NO: 95 - protein, 7 aa, synthetic construct
WASTRKS

SEQ ID NO: 96 - protein, 9 aa, synthetic construct
QQYYGIPLT

SEQ ID NO: 97 - protein, 7 aa, synthetic construct
SNSAAWN

SEQ ID NO: 98 - protein, 18 aa, synthetic construct
RTYYRSKWYNDYAVSVKS

SEQ ID NO: 99 - protein, 8 aa, synthetic construct
GGAAVFDY

SEQ ID NO: 100 - protein, 17 aa, synthetic construct
KSSQSILYSSNNKNYLA

SEQ ID NO: 101 - protein, 7 aa, synthetic construct
WASTRGS

SEQ ID NO: 102 - protein, 9 aa, synthetic construct
QQYYSTPLT

SEQ ID NO: 103 - protein, 7 aa, synthetic construct
SSSAAWN

SEQ ID NO: 104 - protein, 18 aa, synthetic construct
RTYYRSKWYNDYAESVKS

SEQ ID NO: 105 - protein, 15 aa, synthetic construct
RLTIVRGVMRGGMDV

SEQ ID NO: 106 - protein, 17 aa, synthetic construct
KSSQNLLYSANNKDYLA

SEQ ID NO: 107 - protein, 7 aa, synthetic construct
WASTRYS

SEQ ID NO: 108 - protein, 9 aa, synthetic construct
QQYYSTPWT

SEQ ID NO: 109 - protein, 7 aa, synthetic construct
SSSAAWN

SEQ ID NO: 110 - protein, 18 aa, synthetic construct
RTFYRSKWYNDYAESVKS

SEQ ID NO: 111 - protein, 15 aa, synthetic construct
RLTIVRGVMRGGMDV

SEQ ID NO: 112 - protein, 17 aa, synthetic construct
KSSQNLLYSANNKDYIA

SEQ ID NO: 113 - protein, 7 aa, synthetic construct
WASIRYS

SEQ ID NO: 114 - protein, 9 aa, synthetic construct
QQYFSTPWT

SEQ ID NO: 115 - protein, 7 aa, synthetic construct
SSSAAWN

SEQ ID NO: 116 - protein, 18 aa, synthetic construct
RTYYRSKWYNDYAESVKS

SEQ ID NO: 117 - protein, 15 aa, synthetic construct
RLTIVRGVMRGGMDV

SEQ ID NO: 118 - protein, 17 aa, synthetic construct
KSSQNLLYSANNKDYLA

SEQ ID NO: 119 - protein, 7 aa, synthetic construct
WASTRYS

SEQ ID NO: 120 - protein, 9 aa, synthetic construct
QQYYSTPWT

SEQ ID NO: 121 - protein, 7 aa, synthetic construct
SSSAAWN

SEQ ID NO: 122 - protein, 18 aa, synthetic construct
RTYYRSKWYNDYAESVKS

SEQ ID NO: 123 - protein, 15 aa, synthetic construct
RLTIVRGVMRGGMDV

SEQ ID NO: 124 - protein, 17 aa, synthetic construct
KSSQNLLYSANNKDYLA

SEQ ID NO: 125 - protein, 7 aa, synthetic construct
WASTRYS

SEQ ID NO: 126 - protein, 9 aa, synthetic construct
QQYYSTPWT

SEQ ID NO: 127 - protein, 17 aa, synthetic construct
WINPNSSGTNYAQKFQG

SEQ ID NO: 128 - protein, 11 aa, synthetic construct
LAPRLRGAFDI

SEQ ID NO: 129 - protein, 11 aa, synthetic construct
PAWRLRGAFDI

SEQ ID NO: 130 - protein, 11 aa, synthetic construct
PAPRLRMAFDI

SEQ ID NO: 131 - protein, 11 aa, synthetic construct
PAPRLRGAYDI

SEQ ID NO: 132 - protein, 13 aa, synthetic construct
SGSSSNIGTKKVS

SEQ ID NO: 133 - protein, 13 aa, synthetic construct
SGSSSNIGNFKVS

SEQ ID NO: 134 - protein, 11 aa, synthetic construct
VTWDSSLRAVV

SEQ ID NO: 135 - protein, 17 aa, synthetic construct
WINPISGGTNYAQKFQG

SEQ ID NO: 136 - protein, 17 aa, synthetic construct
WINPNTGGTNYAQKFQG

SEQ ID NO: 137 - protein, 138 aa, synthetic construct
MDWTWRILFLVAAATGAHSQVQLVQSGAEVKKPGASVKVSCKASGYTFTGYYMHWVRQAPGQGLEWMGWINPNSGGTNYAQKFQGWVTMTRDTSISTAYMELSRLRSDDTAVYYCARGITGTTPFDYWGQGTLVTVSS

SEQ ID NO: 138 - protein, 127 aa, synthetic construct
MRVPAQLLGLLLLWFPGARCDIQMTQSPSSLSASVGDRVTITCRASQGIRNDLGWYQQKPGKAPKRLIYAASSLQSGVPSRFSGSGSGTEFTLTISSLQPEDFATYYYLQHNSYPYTFGQGTKLEIK

SEQ ID NO: 139 - protein, 141 aa, synthetic construct
MDTLCYTLLLLTTPSWVLSQVTLKESGPVLVKPTETLTLTCTVSGFSLSNARMGVSWIRQPPGKALEWLAHIFSNDEKSYSTSLKSRLTISKDTSKSQVVLTMTNMDPVDTATYYCARVLLWFGELYFDYWGQGTLVTVSS

SEQ ID NO: 140 - protein, 127 aa, synthetic construct
MEAPAQLLFLLLLWLPDTTGEIVMTQSPATLSVFPGERATLSCRASQSVSSNLAWYQQKPGQAPRLLIYGASTRATGIPARFSGSGSGTECTLTISSLQSEDFAVYYCQQYNNWPRTFSQGTKVEIK

SEQ ID NO: 141 - protein, 138 aa, synthetic construct
MDWTWRILFLVAAATGAHSQVQLVQSGAEVKKPGASVKVSCKASGYTFTGYYMHWVRQAPGQGLEWMGWINPNSGGTNYAQKFQGWVTMTRDTSISTAYMELRLRSDDTAVYYCARLGTTGYYYFDYWGQGTLVTVSS

SEQ ID NO: 142 - protein, 126 aa, synthetic construct
MLPSQLIGFLLLWVPASRGEIVLTQSPDFQSVTPKEKVTITCRASQSIGSSLHWYQQKPDQSPKLLIKYASQSFSGVPSRFSGSGSGTDFTLTINSLEAEDAATYYCHQSSSLPRTFGQGTKVEIK

SEQ ID NO: 143 - protein, 145 aa, synthetic construct
MDWTWRILFLVAAATGAHSQVQLVQSGAEVKKPGASVKVSCKASGYTFTSNAMHWVRQAPGQRLEWMGWINAGNGNTKYSQKFQGRVTITRDTSASTAYMELSSLRSEDTAVYYCARGYYDILTGYYTTDAFDIWGQGTMVTVSS

SEQ ID NO: 144 - protein, 132 aa, synthetic construct
MRLPAQLLGLLMLWVPGSSGDVVMTQSPLSLPVTLGQPASISCRSSQSLVYSDGNTYLNWFQQRPGQSPRRLIYKVSNRDSGVPDRFSGSGSGTDFTLKITRVEAEDVGVYYCMQGTHWPYTFGQGTKLEIK

SEQ ID NO: 145 - protein, 139 aa, synthetic construct
MDWTWRILFLVAAATGAHSQVQLVQSGAEVKKPGASVKVSCKASGYIFISYAMHWVRQAPGQRLEWMGWINAGNGYTEYSQKFQGRVTITRDTSALTAYMELRSLRSEDTAVYYCARRGYFDWWAFDYWGQGTLVTVSS

SEQ ID NO: 146 - protein, 126 aa, synthetic construct
MLPSQLIGFLLLWVPASRGEIVLTQSPDFQSVTPKEKVTITCRASQSIGSSLHWYQQKPDQSPKLLIKYASQSFSGVPSRFSGSGSGTDFTLTINSLEAEDAATYYCHQSSSLPQTFGQGTKVEIK

SEQ ID NO: 147 - protein, 137 aa, synthetic construct
MKHLWFFLLLVAAPRWVLSQVQLQESGPGLVKPSGTLSLTCAVSGGSISSSNWWSWVRQPPGKGLEWIGEIDHSGTTTYNPSLKSRVTMSVDQSKNQFSLKLSSVTAADTAVYYCARDGSGSYEGYWGQGTLVTVSS

SEQ ID NO: 148 - protein, 127 aa, synthetic construct
MRVLAQLLGLLLLCFPGARCDIQMTQSPSSLSASVGDRVTITCRASQAISNHLAWFQQKPGKAPKSLIYAASSLQSGVPSKFSGSGSGTDFTLTISSLQPEDFATYYCQQYHSYPITFGQGTRLEIK

SEQ ID NO: 149 - protein, 136 aa, synthetic construct
MKHLWFFLLLVAAPRWVLSQVQLQESGPGLVKPSETLSLTCAVSGGSISSSNWWSWVRQPPGKGLEWIGEIYHGVTTYNPSLKSRVTISVDNSKNQFSLKLSSVTAADTAVYYCARDGSGSYEGYWGQGTLVTVSS

SEQ ID NO: 150 - protein, 127 aa, synthetic construct
MRVLAQLLGLLLLCFPGARCDIQMTQSPSSLSASVGDRVTITCRASQDISNYLAWFQQKPGKAPKSLIYAASSLQSGVPSKFSGSGSGTDFTLTISSLQPEDFATYYCQQYHYYPITFGQGTRLEIK

SEQ ID NO: 151 - protein, 133 aa, synthetic construct
MDWTWRILFLVAAATGAHSQVQLVQSGAEVKKPGASVKVSCKASGYTFFSYAMHWVRQAPGQRLEWMGWINAGNGNTKYSQKFQDRVTITRDTSATTAYMELSSLRSEDTAVYYCASWVFDYWGQGTPVTVSS

SEQ ID NO: 152 - protein, 132 aa, synthetic construct
MRLLAQLLGLLMLWVPGSSGDIVMTQTPLSSLVTLGQPASISCRSSQSLVHRDGNTYLSWLQQRPGQPPRLLIYKISNRFFGVPDRFSGSGAGTDFTLKISRVEAEDVGVYYCMQATQFPHTFGQGTKLEIK

SEQ ID NO: 153 - protein, 147 aa, synthetic construct
MSVSFLIFLPVLGLPWGVLSQVQLQQSGPGLVKPSQTLSLTCAISGDSVSSNSAAWNWIRQSPSRGLEWLGRTYYRSKWYNDYAVSVKSRITINPDTSKNQFSLQLNSVTPEDTAVYYCAREGITVGRGVMLYFDLWGRGTLVTVSS

SEQ ID NO: 154 - protein, 132 aa, synthetic construct
MRLPAQLLGLLMLWVPGSSGDVLMTQSPLSLPVTLGQPASISCRSSQSLVYSDGNTHLKWFQQRPGQSPRRLIYKVSKWDSGVPDRVSGSGSGTDFTLKISRVEAEDVGVYYCMQGTHWPPTFGQGTKVEIK

SEQ ID NO: 155 - protein, 120 aa, synthetic construct
QVQLVQSGAEVKKPGASVKVSCKASGYTFTGYYMHWVRQAPGQGLEWMGWINPNSGGTNYAQKFQGRVTMTRDTSISTAYMELSRLRSDDTAVYYCARPAPRLRGAFDIWGQGTLVTVSS

SEQ ID NO: 156 - protein, 110 aa, synthetic construct
QSVVTQPPSVSAAPGQKVTISCSGSSSNIGNKKVSWYQQLPVTAPKLLIYDDNKRPSGIPDRFSGSKSGTSATLGITGLQTGDEADYYCATWDSSLRAVVFGGGTKLTVL

SEQ ID NO: 157 - protein, 136 aa, synthetic construct
MDWTWRILFLVAAATGAHSQVQLVQSGAEVKKPGASVKVSCKASGYTFTSHAVHWVRQAPGQRLEWMGWINAGKGNTKYSQKFQGRVTITRDTSATTAYMELSSLRSEDTAVYYCARGRAVAFDPWGQGTLVTVSS

SEQ ID NO: 158 - protein, 129 aa, synthetic construct
MAWALLLLTLLTQGTGSWARSALTQPPSASGSPGQSVTVSCTGTNSDIGGYNYVSWYKQHPGNAPKLMIYEVNKRPSGVPDRFSGSKSGNTASLTVSGLQTEDEADYYCASYAGDNNLVFGGGTKLTVL

SEQ ID NO: 159 - protein, 140 aa, synthetic construct
MSVSFLIFLPVLGLPWGVLSQVQLQQSGPGLVKPSQTLSLTCAISGDSVSSNSAAWNWIRQSPSRGLEWLGRTYYRSKWYNDYAVSVKSRITINPDTSKNQFSLQLNSVTPEDTAVYYCARGGAAVFDYWGQGTLVTVSS

SEQ ID NO: 160 - protein, 133 aa, synthetic construct
MVLQTQVFISLLLWISGAYGDIVMTQSPDSLAVSLGERATINCKSSQSILYNSNNKNYLAWYQQNPGQPPKLLFYWASTRGSGVPDRFSGSGSGTDFTLTISSLQAEDVAVYYCQQYYSTPLTFGGGTKVEIK

SEQ ID NO: 161 - protein, 143 aa, synthetic construct
MDWTWRILFLVAAATGAHSQVQLVQSGAEVKKPGASVKVSCKASGYTFTGYYMHWVRQAPGQGLEWMGWINPNSGDTNYAQKFQGWVTMTRDTSISTAYMELSRLRSDDTAVYYCARGGVLLYFGELSRFDYWGQGTLVTVSS

SEQ ID NO: 162 - protein, 129 aa, synthetic construct
MAWALLLLTLLTQGTGSWAQSALTQPPSASGSPGQSVAISCTGTSSDVGGYNYVSWYQQHPGKAPQLLIYEVTKRPSGVPDRFSGSKSGNTASLTVSGLQAEDEADYYCASYAGDNNLVFGGGTKLTVL

SEQ ID NO: 163 - protein, 136 aa, synthetic construct
MDWTWRILFLVAAATGAHSQVQLVQSGAEVKKPGASVKLSCKAAGYTFTVNAMHWVRQAPGQGLEWMGWINAGTGKTKYSQKFQGRLTITRDTSASTAYMHLSGLRSEDTAVYYCARGRAVAFDPWGQGTLVTVSS

SEQ ID NO: 164 - protein, 129 aa, synthetic construct
MAWALLLLTLLTQGTGSWAQSALTQPPSASGSPGQSVTISCTGTSSDVGGYDYVSWYQQHPDKAPKLMIYEVNKRPSGVPDRFSGSKSGNTASLTVSGLQAEDEADYYCNSYAGNNNLVFGGGTKLTVL

SEQ ID NO: 165 - protein, 140 aa, synthetic construct
MSVSFLIFLPVLGLPWGVLSQVQLQQSGPGLVKPSQTLSLTCAISGDSVSSNSAAWNWIRQSPSRGLEWLGRTYYKSKWYNDYAVSVKSRMTINPDTSKNQFSLQLNSVTPEDTAVYYCARGGSAVFDYWGQGTLVTVSS

SEQ ID NO: 166 - protein, 133 aa, synthetic construct
MVLQTQVFISLLLWISGAYGDIVMTQSSDSLAVSLGERATINCKSSQSILYSSNNKNYLAWYQQKLGQPPNLLIYWASTRKSGVPDRFSGSGSGTDFTLTISSLQAEDVAVYYCQQYYGLPLTFGGGTKVEIK

SEQ ID NO: 167 - protein, 140 aa, synthetic construct; identical to SEQ ID NO: 165

SEQ ID NO: 168 - protein, 133 aa, synthetic construct
MVLQTQVFISLLLWISGAYGDIVMTQSSDSLAVSLGERATINCKSSQSVLYSSNNKNYLAWYQQKLGQPPNLLIYWASTRKSGVPDRFSGSGSGTDFTLTISSLQAEDVAVYYCQQYYGIPLTFGGGTKVEIK

SEQ ID NO: 169 - protein, 140 aa, synthetic construct; identical to SEQ ID NO: 159

SEQ ID NO: 170 - protein, 133 aa, synthetic construct
MVLQTQVFISLLLWISGAYGDIVMTQSPDSLAVSLGERATINCKSSQSILYSSNNKNYLAWYQQNPGQPPKLLFYWASTRGSGVPDRFSGSGSGTDFTLTISSLQAEDVAVYYCQQYYSTPLTFGGGTKVEIK

SEQ ID NO: 171 - protein, 147 aa, synthetic construct
MSVSFLIFLPVLGLPWGVLSQVQLQQSGPGLVKPSQTLSLTCAISGDSVSSSSAAWNWIRQSPSRGLEWLGRTYYRSKWYNDYAESVKSRITINPDTSKNQFSLQLNSVTPEDTAVYYCARRLTIVRGVMRGGMDVWGQGTTVTVSS

SEQ ID NO: 172 - protein, 133 aa, synthetic construct
MVLQTQVFISLLLWISGASGDIVMTQSPDSLAVSLDERATINCKSSQNLLYSANNKDYLAWYQQKPGQPPKLLIYWASTRYSGIPDRFSGSGSGTDFTLTISSLQAEDVAVYYCQQYYSTPWTFGQGTKVEIK

SEQ ID NO: 173 - protein, 147 aa, synthetic construct
MSVSFLIFLPVLGLPWGVLSQVQLQQSGPGLVKPSQTLSLTCAISGDSVSSSSAAWNWIRQSPSRGLEWLGRTFYRSKWYNDYAESVKSRITINADTSKNQFSLQLNSVTPEDTAVYYCARRLTIVRGVMRGGMDVWGQGTTVTVSS

SEQ ID NO: 174 - protein, 133 aa, synthetic construct
MVLQTQVFISLLLWISGASGDIVMTQSPDSLTGSLDERATINCKSSQNLLYSANNKDYIAWYQQKPGQSPKLLIYWASIRYSGVPDRFSGSGSGTDFTLTISSLQAEDVAVYYCQQYFSTPWTFGQGTKVEIK

SEQ ID NO: 175 - protein, 147 aa, synthetic construct; identical to SEQ ID NO: 171

SEQ ID NO: 176 - protein, 133 aa, synthetic construct
MVLQTQVFISLLLWISGASGDIVMTQSPDSLAVSLDERATINCKSSQNLLYSANNKDYLAWYQQKPGQSPKLLIYWASTRYSGVPDRFSGSGSGTDFTLTISSLQAEDVAVYYCQQYYSTPWTFGQGTKVEIK

SEQ ID NO: 177 - protein, 147 aa, synthetic construct; identical to SEQ ID NO: 171

SEQ ID NO: 178 - protein, 133 aa, synthetic construct; identical to SEQ ID NO: 176